European Patent Application EP 4 775 692 A1, published July 15, 2026. Title: 用于鉴别罗汉果雌株和雄株的SNP标记及鉴别方法. Applicant: 桂林吉福思罗汉果生物技术股份有限公司. The sequence listing filed with the application follows.

SEQUENCE LISTING (4 sequences)

SEQ ID NO: 1 - DNA, 276 bp, synthetic construct
  source 1..276: mol_type = other DNA
attgtcgtcctacctatctacaaaacagcagagccttcaaagtagaagcggctgcttttactggattattagagagagaagaagttgagaaaatgaatgaactgagatttgcttgcatgctstccatccccaatggttgatttaattcgtttggtaggcagagattgtaaaacatataaacgaaatcttttgggacatgataaaaaattaaattttcagttccatgctttgggttgggcccgtcatattcttattcaacacacgtacggggcgcct

SEQ ID NO: 2 - DNA, 40 bp, synthetic construct
  source 1..40: mol_type = other DNA
gaaggtgaccaagttcatgcttcaaccattggggatggag

SEQ ID NO: 3 - DNA, 40 bp, synthetic construct
  source 1..40: mol_type = other DNA
gaaggtcggagtcaacggatttcaaccattggggatggac

SEQ ID NO: 4 - DNA, 23 bp, synthetic construct
  source 1..23: mol_type = other DNA
gtagaagcggctgcttttactgg